European Patent Application EP 4 775 596 A1, published July 15, 2026. Title: 半胱氨酸改造的抗体和免疫缀合物. Applicant: 信达生物制药(苏州)有限公司. The sequence listing filed with the application follows.

SEQUENCE LISTING (68 sequences)

SEQ ID NO: 1 - protein, 103 aa, synthetic construct
ASTKGPSVFPLAPSSKSTSGGTAALGCLVKDYFPEPVTVSWNSGALTSGVHTFPAVLQSSGLYSLSSVVTVPSSSLGTQTYICNVNHKPSNTKVDKKVEPKSC

SEQ ID NO: 2 - protein, 227 aa, synthetic construct
DKTHTCPPCPAPELLGGPSVFLFPPKPKDTLMISRTPEVTCVVVDVSHEDPEVKFNWYVDGVEVHNAKTKPREEQYNSTYRVVSVLTVLHQDWLNGKEYKCKVSNKALPAPIEKTISKAKGQPREPQVYTLPPSRDELTKNQVSLTCLVKGFYPSDIAVEWESNGQPENNYKTTPPVLDSDGSFFLYSKLTVDKSRWQQGNVFSCSVMHEALHNHYTQKSLSLSPGK

SEQ ID NO: 3 - protein, 330 aa, synthetic construct [sequence omitted]

SEQ ID NO: 4 - protein, 224 aa, synthetic construct
PPCPSCPAPEFLGGPSVFLFPPKPKDTLMISRTPEVTCVVVDVSQEDPEVQFNWYVDGVEVHNAKTKPREEQFNSTYRVVSVLTVLHQDWLNGKEYKCKVSNKGLPSSIEKTISKAKGQPREPQVYTLPPSQEEMTKNQVSLTCLVKGFYPSDIAVEWESNGQPENNYKTTPPVLDSDGSFFLYSRLTVDKSRWQEGNVFSCSVMHEALHNHYTQKSLSLSLGK

SEQ ID NO: 5 - protein, 107 aa, synthetic construct [sequence omitted]

SEQ ID NO: 6 - protein, 106 aa, synthetic construct
GQPKAAPSVTLFPPSSEELQANKATLVCLISDFYPGAVTVAWKADSSPVKAGVETTTPSKQSNNKYAASSYLSLTPEQWKSHRSYSCQVTHEGSTVEKTVAPTECS

SEQ ID NO: 7 - protein, 11 aa, synthetic construct
VKAGVCTTTPS

SEQ ID NO: 8 - protein, 11 aa, synthetic construct
TTTPSCQSNNK

SEQ ID NO: 9 - protein, 11 aa, synthetic construct
QESVTCQDSKD

SEQ ID NO: 10 - protein, 11 aa, synthetic construct
KDYFPCPVTVS

SEQ ID NO: 11 - protein, 11 aa, synthetic construct
KDYFPEPVCVS

SEQ ID NO: 12 - protein, 11 aa, synthetic construct
CLLNCFYPREA

SEQ ID NO: 13 - protein, 11 aa, synthetic construct
NAKTCPREEQY

SEQ ID NO: 14 - protein, 11 aa, synthetic construct
ESVTEQCSKDS

SEQ ID NO: 15 - protein, 12 aa, synthetic construct
GLSSPCTKSFNR

SEQ ID NO: 16 - protein, 106 aa, synthetic construct
GQPKAAPSVTLFPPSSEELQANKATLVCLISDFYPGAVTVAWKADSSPVKAGVCTTTPSKQSNNKYAASSYLSLTPEQWKSHRSYSCQVTHEGSTVEKTVAPTECS

SEQ ID NO: 17 - protein, 106 aa, synthetic construct
GQPKAAPSVTLFPPSSEELQANKATLVCLISDFYPGAVTVAWKADSSPVKAGVETTTPSCQSNNKYAASSYLSLTPEQWKSHRSYSCQVTHEGSTVEKTVAPTECS

SEQ ID NO: 18 - protein, 106 aa, synthetic construct
GQPKAAPSVTLFPPSSEELQANKATLVCLISDFYPGAVTVAWKADSSPVKAGVCTTTPSCQSNNKYAASSYLSLTPEQWKSHRSYSCQVTHEGSTVEKTVAPTECS

SEQ ID NO: 19 - protein, 107 aa, synthetic construct
RTVAAPSVFIFPPSDEQLKSGTASVVCLLNCFYPREAKVQWKVDNALQSGNSQESVTEQDSKDSTYSLSSTLTLSKADYEKHKVYACEVTHQGLSSPVTKSFNRGEC

SEQ ID NO: 20 - protein, 107 aa, synthetic construct
RTVAAPSVFIFPPSDEQLKSGTASVVCLLNNFYPREAKVQWKVDNALQSGNSQESVTCQDSKDSTYSLSSTLTLSKADYEKHKVYACEVTHQGLSSPVTKSFNRGEC

SEQ ID NO: 21 - protein, 107 aa, synthetic construct
RTVAAPSVFIFPPSDEQLKSGTASVVCLLNNFYPREAKVQWKVDNALQSGNSQESVTEQCSKDSTYSLSSTLTLSKADYEKHKVYACEVTHQGLSSPVTKSFNRGEC

SEQ ID NO: 22 - protein, 103 aa, synthetic construct
ASTKGPSVFPLAPSSKSTSGGTAALGCLVKDYFPCPVTVSWNSGALTSGVHTFPAVLQSSGLYSLSSVVTVPSSSLGTQTYICNVNHKPSNTKVDKKVEPKSC

SEQ ID NO: 23 - protein, 103 aa, synthetic construct
ASTKGPSVFPLAPSSKSTSGGTAALGCLVKDYFPEPVCVSWNSGALTSGVHTFPAVLQSSGLYSLSSVVTVPSSSLGTQTYICNVNHKPSNTKVDKKVEPKSC

SEQ ID NO: 24 - protein, 227 aa, synthetic construct
DKTHTCPPCPAPELLGGPSVFLFPPKPKDTLMISRTPEVTCVVVDVSHEDPEVKFNWYVDGVEVHNAKTCPREEQYNSTYRVVSVLTVLHQDWLNGKEYKCKVSNKALPAPIEKTISKAKGQPREPQVYTLPPSRDELTKNQVSLTCLVKGFYPSDIAVEWESNGQPENNYKTTPPVLDSDGSFFLYSKLTVDKSRWQQGNVFSCSVMHEALHNHYTQKSLSLSPGK

SEQ ID NO: 25 - protein, 330 aa, synthetic construct
ASTKGPSVFPLAPSSKSTSGGTAALGCLVKDYFPCPVTVSWNSGALTSGVHTFPAVLQSSGLYSLSSVVTVPSSSLGTQTYICNVNHKPSNTKVDKKVEPKSCDKTHTCPPCPAPELLGGPSVFLFPPKPKDTLMISRTPEVTCVVVDVSHEDPEVKFNWYVDGVEVHNAKTKPREEQYNSTYRVVSVLTVLHQDWLNGKEYKCKVSNKALPAPIEKTISKAKGQPREPQVYTLPPSRDELTKNQVSLTCLVKGFYPSDIAVEWESNGQPENNYKTTPPVLDSDGSFFLYSKLTVDKSRWQQGNVFSCSVMHEALHNHYTQKSLSLSPGK

SEQ ID NO: 26 - protein, 330 aa, synthetic construct
ASTKGPSVFPLAPSSKSTSGGTAALGCLVKDYFPEPVCVSWNSGALTSGVHTFPAVLQSSGLYSLSSVVTVPSSSLGTQTYICNVNHKPSNTKVDKKVEPKSCDKTHTCPPCPAPELLGGPSVFLFPPKPKDTLMISRTPEVTCVVVDVSHEDPEVKFNWYVDGVEVHNAKTKPREEQYNSTYRVVSVLTVLHQDWLNGKEYKCKVSNKALPAPIEKTISKAKGQPREPQVYTLPPSRDELTKNQVSLTCLVKGFYPSDIAVEWESNGQPENNYKTTPPVLDSDGSFFLYSKLTVDKSRWQQGNVFSCSVMHEALHNHYTQKSLSLSPGK

SEQ ID NO: 27 - protein, 330 aa, synthetic construct
ASTKGPSVFPLAPSSKSTSGGTAALGCLVKDYFPEPVTVSWNSGALTSGVHTFPAVLQSSGLYSLSSVVTVPSSSLGTQTYICNVNHKPSNTKVDKKVEPKSCDKTHTCPPCPAPELLGGPSVFLFPPKPKDTLMISRTPEVTCVVVDVSHEDPEVKFNWYVDGVEVHNAKTCPREEQYNSTYRVVSVLTVLHQDWLNGKEYKCKVSNKALPAPIEKTISKAKGQPREPQVYTLPPSRDELTKNQVSLTCLVKGFYPSDIAVEWESNGQPENNYKTTPPVLDSDGSFFLYSKLTVDKSRWQQGNVFSCSVMHEALHNHYTQKSLSLSPGK

SEQ ID NO: 28 - protein, 17 aa, synthetic construct
VKAGVCTTTPSCQSNNK

SEQ ID NO: 29 - protein, 11 aa, synthetic construct
VKAGVETTTPS

SEQ ID NO: 30 - protein, 11 aa, synthetic construct
TTTPSKQSNNK

SEQ ID NO: 31 - protein, 11 aa, synthetic construct
QESVTEQDSKD

SEQ ID NO: 32 - protein, 11 aa, synthetic construct
KDYFPEPVTVS

SEQ ID NO: 33 - protein, 11 aa, synthetic construct
KDYFPEPVTVS

SEQ ID NO: 34 - protein, 11 aa, synthetic construct
CLLNNFYPREA

SEQ ID NO: 35 - protein, 11 aa, synthetic construct
NAKTKPREEQY

SEQ ID NO: 36 - protein, 11 aa, synthetic construct
ESVTEQDSKDS

SEQ ID NO: 37 - protein, 12 aa, synthetic construct
GLSSPVTKSFNR

SEQ ID NO: 38 - protein, 236 aa, synthetic construct
MDFQVQIISFLLISASVIMSRGDIQMTQSPSSLSASVGDRVTITCRASQSISSYLNWYQQKPGKAPKLLIYAASSLQSGVPSRFSGSGSGTDFTLTISSLQPEDFATYYCQQADLPAFAFGGGTKVEIKRTVAAPSVFIFPPSDEQLKSGTASVVCLLNNFYPREAKVQWKVDNALQSGNSQESVTEQDSKDSTYSLSSTLTLSKADYEKHKVYACEVTHQGLSSPVTKSFNRGEC

SEQ ID NO: 39 - protein, 468 aa, synthetic construct
MGWSLILLFLVAVATRVLSEVRLLESGGGLVQPGGSLRLSCAASGFTFSNYAMGWVRQAPGKGLEWVSAISGSGGSTYYADSVKGRFTTSRDDSKNALYLQMNSLRAEDTAVYYCARGGPGWYAADVWGQGTTVTVSSASTKGPSVFPLAPSSKSTSGGTAALGCLVKDYFPEPVTVSWNSGALTSGVHTFPAVLQSSGLYSLSSVVTVPSSSLGTQTYICNVNHKPSNTKVDKKAEPKSCDKTHTCPPCPAPELLGGPSVFLFPPKPKDTLMISRTPEVTCVVVDVSHEDPEVKFNWYVDGVEVHNAKTKPREEQYNSTYRVVSVLTVLHQDWLNGKEYKCKVSNKALPAPIEKTISKAKGQPREPQVYTLPPSRDELTKNQVSLTCLVKGFYPSDIAVEWESNGQPENNYKTTPPVLDSDGSFFLYSKLTVDKSRWQQGNVFSCSVMHEALHNHYTQKSLSLSPGK

SEQ ID NO: 40 - protein, 11 aa, synthetic construct
QSGNSCESVTE

SEQ ID NO: 41 - protein, 11 aa, synthetic construct
ESVTECDSKDS

SEQ ID NO: 42 - protein, 16 aa, synthetic construct
SGNSCESVTECDSKDS

SEQ ID NO: 43 - protein, 107 aa, synthetic construct
RTVAAPSVFIFPPSDEQLKSGTASVVCLLNNFYPREAKVQWKVDNALQSGNSCESVTEQDSKDSTYSLSSTLTLSKADYEKHKVYACEVTHQGLSSPVTKSFNRGEC

SEQ ID NO: 44 - protein, 107 aa, synthetic construct
RTVAAPSVFIFPPSDEQLKSGTASVVCLLNNFYPREAKVQWKVDNALQSGNSQESVTECDSKDSTYSLSSTLTLSKADYEKHKVYACEVTHQGLSSPVTKSFNRGEC

SEQ ID NO: 45 - protein, 107 aa, synthetic construct
RTVAAPSVFIFPPSDEQLKSGTASVVCLLNNFYPREAKVQWKVDNALQSGNSCESVTECDSKDSTYSLSSTLTLSKADYEKHKVYACEVTHQGLSSPVTKSFNRGEC

SEQ ID NO: 46 - protein, 107 aa, synthetic construct
RTCAAPSVFIFPPSDEQLKSGTASVVCLLNNFYPREAKVQWKVDNALQSGNSQESVTEQDSKDSTYSLSSTLTLSKADYEKHKVYACEVTHQGLSSPVTKSFNRGEC

SEQ ID NO: 47 - protein, 330 aa, synthetic construct
CSTKGPSVFPLAPSSKSTSGGTAALGCLVKDYFPEPVTVSWNSGALTSGVHTFPAVLQSSGLYSLSSVVTVPSSSLGTQTYICNVNHKPSNTKVDKKVEPKSCDKTHTCPPCPAPELLGGPSVFLFPPKPKDTLMISRTPEVTCVVVDVSHEDPEVKFNWYVDGVEVHNAKTKPREEQYNSTYRVVSVLTVLHQDWLNGKEYKCKVSNKALPAPIEKTISKAKGQPREPQVYTLPPSRDELTKNQVSLTCLVKGFYPSDIAVEWESNGQPENNYKTTPPVLDSDGSFFLYSKLTVDKSRWQQGNVFSCSVMHEALHNHYTQKSLSLSPGK

SEQ ID NO: 48 - protein, 330 aa, synthetic construct
ASTKGPSVFPLAPSSKSTSGGTAALGCLVKDYFPEPVTVSWNSGALTSGVHTFPAVLQSSGLYSLSSVVTVPSSSLGTQTYICNVNHKPSNTKVDKKVEPKSCDKTHTCPPCPAPELLGGPCVFLFPPKPKDTLMISRTPEVTCVVVDVSHEDPEVKFNWYVDGVEVHNAKTKPREEQYNSTYRVVSVLTVLHQDWLNGKEYKCKVSNKALPAPIEKTISKAKGQPREPQVYTLPPSRDELTKNQVSLTCLVKGFYPSDIAVEWESNGQPENNYKTTPPVLDSDGSFFLYSKLTVDKSRWQQGNVFSCSVMHEALHNHYTQKSLSLSPGK

SEQ ID NO: 49 - protein, 330 aa, synthetic construct
ASTKGPSVFPLAPSSKSTSGGTAALGCLVKDYFPEPVTVSWNSGALTSGVHTFPAVLQSSGLYSLSSVVTVPSSSLGTQTYICNVNHKPSNTKVDKKVEPKSCDKTHTCPPCPAPELLGGPSVFLFPPKPKDTLMISRTPEVTCVVVDVSHEDPEVKFNWYVDGVEVHNAKTKPREEQYNSTYRVVSVLTVLHQDWLNGKEYKCKVSNKALPAPIEKTISKAKGQPREPQVYTLPPSRDELTKNQVSLTCLVKGFYPSDIAVEWESNGQPENNYKTTPPVLDSDGSFFLYSKLTVDKSRWQQGNVFSCSVMHEALHNHYTQKSLCLSPGK

SEQ ID NO: 50 - protein, 330 aa, synthetic construct
CSTKGPSVFPLAPSSKSTSGGTAALGCLVKDYFPEPVTVSWNSGALTSGVHTFPAVLQSSGLYSLSSVVTVPSSSLGTQTYICNVNHKPSNTKVDKKVEPKSCDKTHTCPPCPAPELLGGPCVFLFPPKPKDTLMISRTPEVTCVVVDVSHEDPEVKFNWYVDGVEVHNAKTKPREEQYNSTYRVVSVLTVLHQDWLNGKEYKCKVSNKALPAPIEKTISKAKGQPREPQVYTLPPSRDELTKNQVSLTCLVKGFYPSDIAVEWESNGQPENNYKTTPPVLDSDGSFFLYSKLTVDKSRWQQGNVFSCSVMHEALHNHYTQKSLSLSPGK

SEQ ID NO: 51 - protein, 330 aa, synthetic construct
CSTKGPSVFPLAPSSKSTSGGTAALGCLVKDYFPEPVTVSWNSGALTSGVHTFPAVLQSSGLYSLSSVVTVPSSSLGTQTYICNVNHKPSNTKVDKKVEPKSCDKTHTCPPCPAPELLGGPSVFLFPPKPKDTLMISRTPEVTCVVVDVSHEDPEVKFNWYVDGVEVHNAKTKPREEQYNSTYRVVSVLTVLHQDWLNGKEYKCKVSNKALPAPIEKTISKAKGQPREPQVYTLPPSRDELTKNQVSLTCLVKGFYPSDIAVEWESNGQPENNYKTTPPVLDSDGSFFLYSKLTVDKSRWQQGNVFSCSVMHEALHNHYTQKSLCLSPGK

SEQ ID NO: 52 - protein, 330 aa, synthetic construct
ASTKGPSVFPLAPSSKSTSGGTAALGCLVKDYFPEPVTVSWNSGALTSGVHTFPAVLQSSGLYSLSSVVTVPSSSLGTQTYICNVNHKPSNTKVDKKVEPKSCDKTHTCPPCPAPELLGGPCVFLFPPKPKDTLMISRTPEVTCVVVDVSHEDPEVKFNWYVDGVEVHNAKTKPREEQYNSTYRVVSVLTVLHQDWLNGKEYKCKVSNKALPAPIEKTISKAKGQPREPQVYTLPPSRDELTKNQVSLTCLVKGFYPSDIAVEWESNGQPENNYKTTPPVLDSDGSFFLYSKLTVDKSRWQQGNVFSCSVMHEALHNHYTQKSLCLSPGK

SEQ ID NO: 53 - protein, 11 aa, synthetic construct
QSGNSQESVTE

SEQ ID NO: 54 - protein, 11 aa, synthetic construct
ESVTEQDSKDS

SEQ ID NO: 55 - protein, 12 aa, synthetic construct
RTVAAPSVFIFP

SEQ ID NO: 56 - protein, 11 aa, synthetic construct
LLGGPSVFLFP

SEQ ID NO: 57 - protein, 11 aa, synthetic construct
ASTKGPSVFPL

SEQ ID NO: 58 - protein, 11 aa, synthetic construct
TQKSLSLSPGK

SEQ ID NO: 59 - protein, 11 aa, synthetic construct
KGFYPSDIAVE

SEQ ID NO: 60 - protein, 214 aa, synthetic construct
DIQMTQSPSSLSASVGDRVTITCRASQDVNTAVAWYQQKPGKAPKLLIYSASFLYSGVPSRFSGSRSGTDFTLTISSLQPEDFATYYCQQHYTTPPTFGQGTKVEIKRTVAAPSVFIFPPSDEQLKSGTASVVCLLNNFYPREAKVQWKVDNALQSGNSCESVTECDSKDSTYSLSSYLTLSKADYEKHKVYACEVTHQGLSSPVTKSFNRGEC

SEQ ID NO: 61 - protein, 330 aa, synthetic construct
ASTKGPSVFPLAPSSKSTSGGTAALGCLVKDYFPEPVTVSWNSGALTSGVHTFPAVLQSSGLYSLSSVVTVPSSSLGTQTYICNVNHKPSNTKVDKKVEPKSCDKTHTCPPCPAPELLGGPSVFLFPPKPKDTLMISRTPEVTCVVVDVSHEDPEVKFNWYVDGVEVHNAKTKPREEQYNSTYRVVSVLTVLHQDWLNGKEYKCKVSNKALPAPIEKTISKAKGQPREPQVYTLPPSRDELTKNQVSLTCLVKGFYPCDIAVEWESNGQPENNYKTTPPVLDSDGSFFLYSKLTVDKSRWQQGNVFSCSVMHEALHNHYTQKSLSLSPGK

SEQ ID NO: 62 - protein, 20 aa, synthetic construct
SCESVTECDSKDSTYSLSSY

SEQ ID NO: 63 - protein, 227 aa, synthetic construct
DKTHTCPPCPAPELLGGPSVFLFPPKPKDTLMISRTPEVTCVVVDVSHEDPEVKFNWYVDGVEVHNAKTKPREEQYNSTYRVVSVLTVLHQDWLNGKEYKCKVSNKALPAPIEKTISKAKGQPREPQVYTLPPSRDELTKNQVSLTCLVKGFYPCDIAVEWESNGQPENNYKTTPPVLDSDGSFFLYSKLTVDKSRWQQGNVFSCSVMHEALHNHYTQKSLSLSPGK

SEQ ID NO: 64 - protein, 330 aa, synthetic construct
ASTKGPSVFPLAPSSKSTSGGTAALGCLVKDYFPEPVTVSWNSGALTSGVHTFPAVLQSSGLYSLSSVVTVPSSSLGTQTYICNVNHKPSNTKVDKKVEPKSCDKTHTCPPCPAPELLGGPCVFLFPPKPKDTLMISRTPEVTCVVVDVSHEDPEVKFNWYVDGVEVHNAKTKPREEQYNSTYRVVSVLTVLHQDWLNGKEYKCKVSNKALPAPIEKTISKAKGQPREPQVYTLPPSRDELTKNQVSLTCLVKGFYPCDIAVEWESNGQPENNYKTTPPVLDSDGSFFLYSKLTVDKSRWQQGNVFSCSVMHEALHNHYTQKSLSLSPGK

SEQ ID NO: 65 - protein, 227 aa, synthetic construct
DKTHTCPPCPAPELLGGPCVFLFPPKPKDTLMISRTPEVTCVVVDVSHEDPEVKFNWYVDGVEVHNAKTKPREEQYNSTYRVVSVLTVLHQDWLNGKEYKCKVSNKALPAPIEKTISKAKGQPREPQVYTLPPSRDELTKNQVSLTCLVKGFYPCDIAVEWESNGQPENNYKTTPPVLDSDGSFFLYSKLTVDKSRWQQGNVFSCSVMHEALHNHYTQKSLSLSPGK

SEQ ID NO: 66 - protein, 11 aa, synthetic construct
ESVTECDSKDS

SEQ ID NO: 67 - protein, 11 aa, synthetic construct
KGFYPCDIAVE

SEQ ID NO: 68 - protein, 11 aa, synthetic construct
LLGGPCVFLFP